European Patent Application EP 4 233 917 A1, published August 30, 2023. Title: ANTI-INFECTIVE CONJUGATE FOR USE IN THE TREATMENT OF ZIKA VIRUS INFECTION. Applicant: Universitat Pompeu Fabra INSTITUTO DE MEDICINA MOLECULAR JOÃO LOBO ANTUNES Instituto de Bioquímica Médica Leopoldo de Meis Faculdade de Medicina da Universidade de Lisboa. The sequence listing filed with the application follows.

SEQUENCE LISTING (4 sequences)

SEQ ID NO: 1 - protein, 10 aa, Dengue virus type 2
VQQLTKRFSL

SEQ ID NO: 2 - protein, 7 aa, Artificial Sequence
  SEQ ID NO3
SGTQEEY

SEQ ID NO: 3 - protein, 8 aa, Artificial Sequence
  SEQ ID NO4
SGTQEEYK

SEQ ID NO: 4 - protein, 11 aa, Artificial Sequence
  SEQ ID NO2
VQQLTKRFSLK